European Patent Application EP 4 230 651 A1, published August 23, 2023. Title: Testosterone-specific Affibody and Uses thereof. Applicant: INSSEN Inc. The sequence listing filed with the application follows.

SEQUENCE LISTING (70 sequences)

SEQ ID NO: 1 - protein, 58 aa, Artificial Sequence
  T26 (Parental)
VDNKFNKEMVQAMREISYLPNLNHTQIRAFIWVLFDDPSQSANLLAEAKKLNDAQAPK

SEQ ID NO: 2 - protein, 58 aa, Artificial Sequence
  T26-Q11A
VDNKFNKEMVAAMREISYLPNLNHTQIRAFIWVLFDDPSQSANLLAEAKKLNDAQAPK

SEQ ID NO: 3 - protein, 58 aa, Artificial Sequence
  T26-S17A
VDNKFNKEMVQAMREIAYLPNLNHTQIRAFIWVLFDDPSQSANLLAEAKKLNDAQAPK

SEQ ID NO: 4 - protein, 58 aa, Artificial Sequence
  T26-T25A
VDNKFNKEMVQAMREISYLPNLNHAQIRAFIWVLFDDPSQSANLLAEAKKLNDAQAPK

SEQ ID NO: 5 - protein, 58 aa, Artificial Sequence
  T26-T25R
VDNKFNKEMVQAMREISYLPNLNHRQIRAFIWVLFDDPSQSANLLAEAKKLNDAQAPK

SEQ ID NO: 6 - protein, 58 aa, Artificial Sequence
  T26-T25H
VDNKFNKEMVQAMREISYLPNLNHHQIRAFIWVLFDDPSQSANLLAEAKKLNDAQAPK

SEQ ID NO: 7 - protein, 58 aa, Artificial Sequence
  T26-T25K
VDNKFNKEMVQAMREISYLPNLNHKQIRAFIWVLFDDPSQSANLLAEAKKLNDAQAPK

SEQ ID NO: 8 - protein, 58 aa, Artificial Sequence
  T26-T25D
VDNKFNKEMVQAMREISYLPNLNHDQIRAFIWVLFDDPSQSANLLAEAKKLNDAQAPK

SEQ ID NO: 9 - protein, 58 aa, Artificial Sequence
  T26-T25E
VDNKFNKEMVQAMREISYLPNLNHEQIRAFIWVLFDDPSQSANLLAEAKKLNDAQAPK

SEQ ID NO: 10 - protein, 58 aa, Artificial Sequence
  T26-T25S
VDNKFNKEMVQAMREISYLPNLNHSQIRAFIWVLFDDPSQSANLLAEAKKLNDAQAPK

SEQ ID NO: 11 - protein, 58 aa, Artificial Sequence
  T26-T25N
VDNKFNKEMVQAMREISYLPNLNHNQIRAFIWVLFDDPSQSANLLAEAKKLNDAQAPK

SEQ ID NO: 12 - protein, 58 aa, Artificial Sequence
  T26-T25Q
VDNKFNKEMVQAMREISYLPNLNHQQIRAFIWVLFDDPSQSANLLAEAKKLNDAQAPK

SEQ ID NO: 13 - protein, 58 aa, Artificial Sequence
  T26-T25C
VDNKFNKEMVQAMREISYLPNLNHCQIRAFIWVLFDDPSQSANLLAEAKKLNDAQAPK

SEQ ID NO: 14 - protein, 58 aa, Artificial Sequence
  T26-T25G
VDNKFNKEMVQAMREISYLPNLNHGQIRAFIWVLFDDPSQSANLLAEAKKLNDAQAPK

SEQ ID NO: 15 - protein, 58 aa, Artificial Sequence
  T26-T25P
VDNKFNKEMVQAMREISYLPNLNHPQIRAFIWVLFDDPSQSANLLAEAKKLNDAQAPK

SEQ ID NO: 16 - protein, 58 aa, Artificial Sequence
  T26-T25V
VDNKFNKEMVQAMREISYLPNLNHVQIRAFIWVLFDDPSQSANLLAEAKKLNDAQAPK

SEQ ID NO: 17 - protein, 58 aa, Artificial Sequence
  T26-T25I
VDNKFNKEMVQAMREISYLPNLNHIQIRAFIWVLFDDPSQSANLLAEAKKLNDAQAPK

SEQ ID NO: 18 - protein, 58 aa, Artificial Sequence
  T26-T25L
VDNKFNKEMVQAMREISYLPNLNHLQIRAFIWVLFDDPSQSANLLAEAKKLNDAQAPK

SEQ ID NO: 19 - protein, 58 aa, Artificial Sequence
  T26-T25F
VDNKFNKEMVQAMREISYLPNLNHFQIRAFIWVLFDDPSQSANLLAEAKKLNDAQAPK

SEQ ID NO: 20 - protein, 58 aa, Artificial Sequence
  T26-T25Y
VDNKFNKEMVQAMREISYLPNLNHYQIRAFIWVLFDDPSQSANLLAEAKKLNDAQAPK

SEQ ID NO: 21 - protein, 58 aa, Artificial Sequence
  T26-T25M
VDNKFNKEMVQAMREISYLPNLNHMQIRAFIWVLFDDPSQSANLLAEAKKLNDAQAPK

SEQ ID NO: 22 - protein, 58 aa, Artificial Sequence
  T26-T25W
VDNKFNKEMVQAMREISYLPNLNHWQIRAFIWVLFDDPSQSANLLAEAKKLNDAQAPK

SEQ ID NO: 23 - DNA, 174 bp, Artificial Sequence
  T26 (Parental)
gtggacaacaagttcaacaaggagatggttcaggccatgcgtgagatttcttacctgcccaacctgaaccatacgcagatccgtgccttcatttgggttctgttcgacgacccttcccagtccgccaacctgctggccgaggccaagaagctgaacgacgcccaggctcccaag

SEQ ID NO: 24 - DNA, 174 bp, Artificial Sequence
  T26-Q11A
gtggacaacaagttcaacaaggagatggttgctgccatgcgtgagatttcttacctgcccaacctgaaccatacgcagatccgtgccttcatttgggttctgttcgacgacccttcccagtccgccaacctgctggccgaggccaagaagctgaacgacgcccaggctcccaag

SEQ ID NO: 25 - DNA, 174 bp, Artificial Sequence
  T26-S17A
gtggacaacaagttcaacaaggagatggttcaggccatgcgtgagattgcttacctgcccaacctgaaccatacgcagatccgtgccttcatttgggttctgttcgacgacccttcccagtccgccaacctgctggccgaggccaagaagctgaacgacgcccaggctcccaag

SEQ ID NO: 26 - DNA, 174 bp, Artificial Sequence
  T26-T25A
gtggacaacaagttcaacaaggagatggttcaggccatgcgtgagatttcttacctgcccaacctgaaccatgctcagatccgtgccttcatttgggttctgttcgacgacccttcccagtccgccaacctgctggccgaggccaagaagctgaacgacgcccaggctcccaag

SEQ ID NO: 27 - DNA, 174 bp, Artificial Sequence
  T26-T25R
gtggacaacaagttcaacaaggagatggttcaggccatgcgtgagatttcttacctgcccaacctgaaccataggcagatccgtgccttcatttgggttctgttcgacgacccttcccagtccgccaacctgctggccgaggccaagaagctgaacgacgcccaggctcccaag

SEQ ID NO: 28 - DNA, 174 bp, Artificial Sequence
  T26-T25H
gtggacaacaagttcaacaaggagatggttcaggccatgcgtgagatttcttacctgcccaacctgaaccatcatcagatccgtgccttcatttgggttctgttcgacgacccttcccagtccgccaacctgctggccgaggccaagaagctgaacgacgcccaggctcccaag

SEQ ID NO: 29 - DNA, 174 bp, Artificial Sequence
  T26-T25K
gtggacaacaagttcaacaaggagatggttcaggccatgcgtgagatttcttacctgcccaacctgaaccataagcagatccgtgccttcatttgggttctgttcgacgacccttcccagtccgccaacctgctggccgaggccaagaagctgaacgacgcccaggctcccaag

SEQ ID NO: 30 - DNA, 174 bp, Artificial Sequence
  T26-T25D
gtggacaacaagttcaacaaggagatggttcaggccatgcgtgagatttcttacctgcccaacctgaaccatgatcagatccgtgccttcatttgggttctgttcgacgacccttcccagtccgccaacctgctggccgaggccaagaagctgaacgacgcccaggctcccaag

SEQ ID NO: 31 - DNA, 174 bp, Artificial Sequence
  T26-T25E
gtggacaacaagttcaacaaggagatggttcaggccatgcgtgagatttcttacctgcccaacctgaaccatgagcagatccgtgccttcatttgggttctgttcgacgacccttcccagtccgccaacctgctggccgaggccaagaagctgaacgacgcccaggctcccaag

SEQ ID NO: 32 - DNA, 174 bp, Artificial Sequence
  T26-T25S
gtggacaacaagttcaacaaggagatggttcaggccatgcgtgagatttcttacctgcccaacctgaaccatagtcagatccgtgccttcatttgggttctgttcgacgacccttcccagtccgccaacctgctggccgaggccaagaagctgaacgacgcccaggctcccaag

SEQ ID NO: 33 - DNA, 174 bp, Artificial Sequence
  T26-T25N
gtggacaacaagttcaacaaggagatggttcaggccatgcgtgagatttcttacctgcccaacctgaaccataatcagatccgtgccttcatttgggttctgttcgacgacccttcccagtccgccaacctgctggccgaggccaagaagctgaacgacgcccaggctcccaag

SEQ ID NO: 34 - DNA, 174 bp, Artificial Sequence
  T26-T25Q
gtggacaacaagttcaacaaggagatggttcaggccatgcgtgagatttcttacctgcccaacctgaaccatcagcagatccgtgccttcatttgggttctgttcgacgacccttcccagtccgccaacctgctggccgaggccaagaagctgaacgacgcccaggctcccaag

SEQ ID NO: 35 - DNA, 174 bp, Artificial Sequence
  T26-T25C
gtggacaacaagttcaacaaggagatggttcaggccatgcgtgagatttcttacctgcccaacctgaaccattgtcagatccgtgccttcatttgggttctgttcgacgacccttcccagtccgccaacctgctggccgaggccaagaagctgaacgacgcccaggctcccaag

SEQ ID NO: 36 - DNA, 174 bp, Artificial Sequence
  T26-T25G
gtggacaacaagttcaacaaggagatggttcaggccatgcgtgagatttcttacctgcccaacctgaaccatggtcagatccgtgccttcatttgggttctgttcgacgacccttcccagtccgccaacctgctggccgaggccaagaagctgaacgacgcccaggctcccaag

SEQ ID NO: 37 - DNA, 174 bp, Artificial Sequence
  T26-T25P
gtggacaacaagttcaacaaggagatggttcaggccatgcgtgagatttcttacctgcccaacctgaaccatcctcagatccgtgccttcatttgggttctgttcgacgacccttcccagtccgccaacctgctggccgaggccaagaagctgaacgacgcccaggctcccaag

SEQ ID NO: 38 - DNA, 174 bp, Artificial Sequence
  T26-T25V
gtggacaacaagttcaacaaggagatggttcaggccatgcgtgagatttcttacctgcccaacctgaaccatgtgcagatccgtgccttcatttgggttctgttcgacgacccttcccagtccgccaacctgctggccgaggccaagaagctgaacgacgcccaggctcccaag

SEQ ID NO: 39 - DNA, 174 bp, Artificial Sequence
  T26-T25I
gtggacaacaagttcaacaaggagatggttcaggccatgcgtgagatttcttacctgcccaacctgaaccatattcagatccgtgccttcatttgggttctgttcgacgacccttcccagtccgccaacctgctggccgaggccaagaagctgaacgacgcccaggctcccaag

SEQ ID NO: 40 - DNA, 174 bp, Artificial Sequence
  T26-T25L
gtggacaacaagttcaacaaggagatggttcaggccatgcgtgagatttcttacctgcccaacctgaaccatcttcagatccgtgccttcatttgggttctgttcgacgacccttcccagtccgccaacctgctggccgaggccaagaagctgaacgacgcccaggctcccaag

SEQ ID NO: 41 - DNA, 174 bp, Artificial Sequence
  T26-T25F
gtggacaacaagttcaacaaggagatggttcaggccatgcgtgagatttcttacctgcccaacctgaaccattttcagatccgtgccttcatttgggttctgttcgacgacccttcccagtccgccaacctgctggccgaggccaagaagctgaacgacgcccaggctcccaag

SEQ ID NO: 42 - DNA, 174 bp, Artificial Sequence
  T26-T25Y
gtggacaacaagttcaacaaggagatggttcaggccatgcgtgagatttcttacctgcccaacctgaaccattatcagatccgtgccttcatttgggttctgttcgacgacccttcccagtccgccaacctgctggccgaggccaagaagctgaacgacgcccaggctcccaag

SEQ ID NO: 43 - DNA, 174 bp, Artificial Sequence
  T26-T25M
gtggacaacaagttcaacaaggagatggttcaggccatgcgtgagatttcttacctgcccaacctgaaccatatgcagatccgtgccttcatttgggttctgttcgacgacccttcccagtccgccaacctgctggccgaggccaagaagctgaacgacgcccaggctcccaag

SEQ ID NO: 44 - DNA, 174 bp, Artificial Sequence
  T26-T25W
gtggacaacaagttcaacaaggagatggttcaggccatgcgtgagatttcttacctgcccaacctgaaccattggcagatccgtgccttcatttgggttctgttcgacgacccttcccagtccgccaacctgctggccgaggccaagaagctgaacgacgcccaggctcccaag

SEQ ID NO: 45 - DNA, 23 bp, Artificial Sequence
  #22 forward
gtgtggaattgtgagcggataac

SEQ ID NO: 46 - DNA, 27 bp, Artificial Sequence
  #24 reverse
atagcccccttattagcgtttgccatc

SEQ ID NO: 47 - DNA, 35 bp, Artificial Sequence
  M9A-forward
caagttcaacaaggaggctgttcaggccatgcgtg

SEQ ID NO: 48 - DNA, 35 bp, Artificial Sequence
  V10A-forward
gttcaacaaggagatggctcaggccatgcgtgaga

SEQ ID NO: 49 - DNA, 36 bp, Artificial Sequence
  Q11A-forward
caacaaggagatggttgctgccatgcgtgagatttc

SEQ ID NO: 50 - DNA, 35 bp, Artificial Sequence
  M13A-forward
ggagatggttcaggccgctcgtgagatttcttacc

SEQ ID NO: 51 - DNA, 35 bp, Artificial Sequence
  R14A-forward
gatggttcaggccatggctgagatttcttacctgc

SEQ ID NO: 52 - DNA, 39 bp, Artificial Sequence
  S17A-forward
caggccatgcgtgagattgcttacctgcccaacctgaac

SEQ ID NO: 53 - DNA, 35 bp, Artificial Sequence
  Y18A-forward
catgcgtgagatttctgctctgcccaacctgaacc

SEQ ID NO: 54 - DNA, 41 bp, Artificial Sequence
  H24A-forward
cttacctgcccaacctgaacgctactcagatccgtgccttc

SEQ ID NO: 55 - DNA, 38 bp, Artificial Sequence
  T25A-forward
ctgcccaacctgaaccatgctcagatccgtgccttcat

SEQ ID NO: 56 - DNA, 41 bp, Artificial Sequence
  I27A-forward
caacctgaaccatactcaggctcgtgccttcatttgggttc

SEQ ID NO: 57 - DNA, 39 bp, Artificial Sequence
  R28A-forward
ctgaaccatactcagatcgctgccttcatttgggttctg

SEQ ID NO: 58 - DNA, 40 bp, Artificial Sequence
  W32A-forward
cagatccgtgccttcattgctgttctgttcgacgaccctt

SEQ ID NO: 59 - DNA, 40 bp, Artificial Sequence
  V33A-forward
gatccgtgccttcatttgggctctgttcgacgacccttcc

SEQ ID NO: 60 - DNA, 37 bp, Artificial Sequence
  F35A-forward
ccttcatttgggttctggctgacgacccttcccagtc

SEQ ID NO: 61 - DNA, 38 bp, Artificial Sequence
  T25NNK-forward
ctgcccaacctgaaccatnnkcagatccgtgccttcat

SEQ ID NO: 62 - DNA, 18 bp, Artificial Sequence
  T25-reverse
atggttcaggttgggcag

SEQ ID NO: 63 - DNA, 34 bp, Artificial Sequence
  forward primer
aattcatatggtggacaacaagttcaacaaggag

SEQ ID NO: 64 - DNA, 31 bp, Artificial Sequence
  reverse primer
ccgctcgagcttgggagcctgggcgtcgttc

SEQ ID NO: 65 - DNA, 64 bp, Artificial Sequence
  reverse (T26-INS001)
ccgctcgagttagcgcaggccatacaccacgctgccgccgccgcccttgggagcctgggcgtcg

SEQ ID NO: 66 - protein, 7 aa, Artificial Sequence
  INS001 (OPN-R)
SVVYGLR

SEQ ID NO: 67 - protein, 79 aa, Artificial Sequence
  T26 expression
MGSSHHHHHHSSGLVPRGSHMVDNKFNKEMVQAMREISYLPNLNHTQIRAFIWVLFDDPSQSANLLAEAKKLNDAQAPK

SEQ ID NO: 68 - DNA, 240 bp, Artificial Sequence
  T26 expression
atgggcagcagccatcatcatcatcatcacagcagcggcctggtgccgcgcggcagccatatggtggacaacaagttcaacaaggagatggttcaggccatgcgtgagatttcttacctgcccaacctgaaccatacgcagatccgtgccttcatttgggttctgttcgacgacccttcccagtccgccaacctgctggccgaggccaagaagctgaacgacgcccaggctcccaagtaa

SEQ ID NO: 69 - protein, 90 aa, Artificial Sequence
  T26-INS001 expression
MGSSHHHHHHSSGLVPRGSHMVDNKFNKEMVQAMREISYLPNLNHTQIRAFIWVLFDDPSQSANLLAEAKKLNDAQAPKGGGGSVVYGLR

SEQ ID NO: 70 - DNA, 273 bp, Artificial Sequence
  T26-INS001 expression
atgggcagcagccatcatcatcatcatcacagcagcggcctggtgccgcgcggcagccatatggtggacaacaagttcaacaaggagatggttcaggccatgcgtgagatttcttacctgcccaacctgaaccatacgcagatccgtgccttcatttgggttctgttcgacgacccttcccagtccgccaacctgctggccgaggccaagaagctgaacgacgcccaggctcccaagggcggcggcggcagcgtggtgtatggcctgcgctaa